European Patent Specification EP 3 265 484 B1, published December 25, 2024. Title: SCFV-FC DIMERS THAT BIND TRANSFORMING GROWTH FACTOR-Beta1 WITH HIGH AFFINITY, AVIDITY AND SPECIFICITY. Applicant: Pan, Clark Qiu, Huawei Bird, Julie. The sequence listing filed with the application follows.

SEQUENCE LISTING (30 sequences)

SEQ ID NO: 1 - protein, 123 aa, Homo sapiens
EVQLVESGGGVVQPGRSLRLSCAASGFTFSSYGMHWVRQAPGKELEWVAVISYDGSIKYYADSVKGRFTISRDNSKNTLYLQMNSLRAEDTAVYYCARTGEYSGYDTDPQYSWGQGTTVTVSS

SEQ ID NO: 2 - protein, 123 aa, Homo sapiens
QVQLVESGGGVVQPGRSLRLSCAASGFTFSSYGMHWVRQAPGKELEWVAVISYDGSIKYYADSVKGRFTISRDNSKNTLYLQMNSLRAEDTAVYYCARTGEYSGYDTPASPDWGQGTTVTVSS

SEQ ID NO: 3 - protein, 15 aa, Artificial Sequence
  Synthetic
SGGGSGGGGSGGGGS

SEQ ID NO: 4 - protein, 15 aa, Artificial Sequence
  Synthetic
GGGGSGGGGSGGGGS

SEQ ID NO: 5 - protein, 107 aa, Homo sapiens
EIVLTQSPSSLSASVGDRVTITCRASQGIGDDLGWYQQKPGKAPILLIYGTSTLQSGVPSRFSGSGSGTDFTLTINSLQPEDFATYYCLQDSNYPLTFGGGTRLEIK

SEQ ID NO: 6 - protein, 107 aa, Homo sapiens
EIVLTQSPSSLSASVGDRVTITCRSSQGIGDDLGWYQQKPGKAPILLIYGTSTLQSGVPSRFSGSGSGTDFTLTINSLQPEDFATYYCLQDSNYPLTFGGGTRLEIK

SEQ ID NO: 7 - protein, 22 aa, Homo sapiens
PKSCDKTHTCPPCPAPELLGGP

SEQ ID NO: 8 - protein, 209 aa, Homo sapiens
SVFLFPPKPKDTLMISRTPEVTCVVVDVSHEDPEVKFNWYVDGVEVHNAKTKPREEQYNSTYRVVSVLTVLHQDWLNGKEYKCKVSNKALPAPIEKTISKAKGQPREPQVYTLPPSRDELTKNQVSLTCLVKGFYPSDIAVEWESNGQPENNYKTTPPVLDSDGSFFLYSKLTVDKSRWQQGNVFSCSVMHEALHNHYTQKSLSLSPGK

SEQ ID NO: 9 - protein, 480 aa, Homo sapiens
EVQLVESGGGVVQPGRSLRLSCAASGFTFSSYGMHWVRQAPGKELEWVAVISYDGSIKYYADSVKGRFTISRDNSKNTLYLQMNSLRAEDTAVYYCARTGEYSGYDTDPQYSWGQGTTVTVSSSGGGSGGGGSGGGGSEIVLTQSPSSLSASVGDRVTITCRSSQGIGDDLGWYQQKPGKAPILLIYGTSTLQSGVPSRFSGSGSGTDFTLTINSLQPEDFATYYCLQDSNYPLTFGGGTRLEIKGGSGPKSCDKTHTCPPCPAPELLGGPSVFLFPPKPKDTLMISRTPEVTCVVVDVSHEDPEVKFNWYVDGVEVHNAKTKPREEQYNSTYRVVSVLTVLHQDWLNGKEYKCKVSNKALPAPIEKTISKAKGQPREPQVYTLPPSRDELTKNQVSLTCLVKGFYPSDIAVEWESNGQPENNYKTTPPVLDSDGSFFLYSKLTVDKSRWQQGNVFSCSVMHEALHNHYTQKSLSLSPGK

SEQ ID NO: 10 - protein, 213 aa, Homo sapiens
EWLTQSPSSLSASVGDRVTITCRASQGIGDDLGWYQQKPGKAPILLIYGTSTLQSGVPSRFSGSGSGTDFTLTINSLQPEDFATYYCLQDSNYPLTFGGGTRLEIKRTVAAPSVFIFPPSDEQLKSGTASVVCLLNNFYPREAKVQWKVDNALQSGNSQESVTEQDSKDSTYSLSSTLTLSKADYEKHKVYACEVTHQGLSSPVTKSFNRGEC

SEQ ID NO: 11 - protein, 450 aa, Homo sapiens
EVQLVESGGGVVQPGRSLRLSCAASGFTFSSYGMHWVRQAPGKELEWVAVISYDGSIKYYADSVKGRFTISRDNSKNTLYLQMNSLRAEDTAVYYCARTGEYSGYDTDPQYSWGQGTTVTVSSASTKGPSVFPLAPCSRSTSESTAALGCLVKDYFPEPVTVSWNSGALTSGVHTFPAVLQSSGLYSLSSVVTVPSSSLGTKTYTCNVDHKPSNTKVDKRVESKYGPPCPSCPAPEFLGGPSVFLFPPKPKDTLMISRTPEVTCVVVDVSQEDPEVQFNWYVDGVEVHNAKTKPREEQFNSTYRVVSVLTVLHQDWLNGKEYKCKVSNKGLPSSIEKTISKAKGQPREPQVYTLPPSQEEMTKNQVSLTCLVKGFYPSDIAVEWESNGQPENNYKTTPPVLDSDGSFFLYSRLTVDKSRWQEGNVFSCSVMHEALHNHYTQKSLSLSLGK

SEQ ID NO: 12 - protein, 245 aa, Homo sapiens
EVQLVESGGGVVQPGRSLRLSCAASGFTFSSYGMHWVRQAPGKELEWVAVISYDGSIKYYADSVKGRFTISRDNSKNTLYLQMNSLRAEDTAVYYCARTGEYSGYDTDPQYSWGQGTTVTVSSSGGGSGGGGSGGGGSEIVLTQSPSSLSASVGDRVTITCRSSQGIGDDLGWYQQKPGKAPILLIYGTSTLQSGVPSRFSGSGSGTDFTLTINSLQPEDFATYYCLQDSNYPLTFGGGTRLEIK

SEQ ID NO: 13 - DNA, 984 bp, Homo sapiens
atgaccatgattacgccaagctttggagccttttttttggagattttcaacgtgaaaaaattattattcgcaattcctttagttgttcctttctatgcggcccagccggccatggccgaggtgcagctggtggagtctgggggaggcgtggtccagcctgggaggtccctgagactctcctgtgcagcctctggattcaccttcagtagctatggcatgcactgggtccgccaggctccaggcaaggagctggagtgggtggcagttatatcatatgatggaagtattaaatactatgcagactccgtgaagggccgattcaccatctccagagacaattccaagaacacgctgtatctgcaaatgaacagcctgagagctgaggacacggctgtgtattactgtgcgcgaactggtgaatatagtggctacgatacggacccccagtactcctgggggcaagggaccacggtcaccgtctcctcaggttcctctggcggtgaaattgtgctgactcagtctccatcctccctgtctgcatctgtaggagacagagtcaccatcacttgccggtcaagtcagggcattggagatgatttgggctggtatcagcagaagccagggaaagcccctatcctcctgatctatggtacatccactttacaaagtggggtcccgtcaaggttcagcggcagtggatctggcacagatttcactctcaccatcaacagcctgcagcctgaagattttgcaacttattactgtctacaagattccaattacccgctcactttcggcggagggacacgactggagattaaacgtgcggccgcacatcatcatcaccatcacggggccgcagaacaaaaactcatctcagaagaggatctgaatggggccgcatagtagctcgagatcaaacgggctagccagccagaactcgccccggaagaccccgaggatgtcgagcaccaccaccaccac

SEQ ID NO: 14 - protein, 262 aa, Homo sapiens
EVQLVESGGGVVQPGRSLRLSCAASGFTESSYGMHWVRQAPGKELEWVAVISYDGSIKYYADSVKGRFTISRDNSKNTLYLQMNSLRAEDTAVYYCARTGEYSGYDTDPQYSWGQGTTVTVSSGSSGGEIVLTQSPSSLSASVGDRVTITCRSSQGIGDDLGWYQQKPGKAPILLIYGTSTLQSGVPSRFSGSGSGTDFTLTINSLQPEDFATYYCLQDSNYPLTFGGGTRLEIKRAAAHHHHHHGAAEQKLISEEDLNGAA

SEQ ID NO: 15 - DNA, 984 bp, Homo sapiens
gaggtgcagctggtggagtctgggggaggcgtggtccagcctgggaggtccctgagactctcctgtgcagcctctggattcaccttcagtagctatggcatgcactgggtccgccaggctccaggcaaggagctggagtgggtggcagttatatcatatgatggaagtattaaatactatgcagactccgtgaagggccgattcaccatctccagagacaattccaagaacacgctgtatctgcaaatgaacagcctgagagctgaggacacggctgtgtattactgtgcgcgaactggtgaatatagtggctacgatacggacccccagtactcctgggggcaagggaccacggtcaccgtctcctcaagtggaggcggttcaggcggaggtggcagcggcggtggcggatcggaaattgtgctgactcagtctccatcctccctgtctgcatctgtaggagacagagtcaccatcacttgccggtcaagtcagggcattggagatgatttgggctggtatcagcagaagccagggaaagcccctatcctcctgatctatggtacatccactttacaaagtggggtcccgtcaaggttcagcggcagtggatctggcacagatttcactctcaccatcaacagcctgcagcctgaagattttgcaacttattactgtctacaagattccaattacccgctcactttcggcggagggacacgactggagattaaacgtgcggccgcacatcatcatcaccatcacggggccgcagaacaaaaactcatctcagaagaggatctgaatggggccgcacccaagcccagtacccccccaggttcttcaggcgaactggaagaactgctgaaacatctgaaagaactgctgaaaggcccgcgtaaaggcgaactggaagaactgctgaaacatctgaaagaactgctgaaaggcggtgcgccgggcggtcatcatcatcaccatcat

SEQ ID NO: 16 - protein, 328 aa, Homo sapiens
EVQLVESGGGVVQPGRSLRLSCAASGFTFSSYGMHWVRQAPGKELEWVAVISYDGSIKYYADSVKGRFTISRDNSKNTLYLQMNSLRAEDTAVYYCARTGEYSGYDTDPQYSWGQGTTVTVSSSGGGSGGGGSGGGGSEIVLTQSPSSLSASVGDRVTITCRSSQGIGDDLGWYQQKPGKAPILLIYGTSTLQSGVPSRFSGSGSGTDFTLTINSLQPEDFATYYCLQDSNYPLTFGGGTRLEIKRAAAHHHHHHGAAEQKLISEEDLNGAAPKPSTPPGSSGELEELLKHLKELLKGPRKGELEELLKHLKELLKGGAPGGHHHHHH

SEQ ID NO: 17 - DNA, 1446 bp, Homo sapiens
gaggtgcagctggtggagtctgggggaggcgtggtccagcctgggaggtccctgagactctcctgtgcagcctctggattcaccttcagtagctatggcatgcactgggtccgccaggctccaggcaaggagctggagtgggtggcagttatatcatatgatggaagtattaaatactatgcagactccgtgaagggccgattcaccatctccagagacaattccaagaacacgctgtatctgcaaatgaacagcctgagagctgaggacacggctgtgtattactgtgcgcgaactggtgaatatagtggctacgatacggacccccagtactcctgggggcaagggaccacggtcaccgtctcctcaagtggaggcggttcaggcggaggtggcagcggcggtggcggatcggaaattgtgctgactcagtctccatcctccctgtctgcatctgtaggagacagagtcaccatcacttgccggtcaagtcagggcattggagatgatttgggctggtatcagcagaagccagggaaagcccctatcctcctgatctatggtacatccactttacaaagtggggtcccgtcaaggttcagcggcagtggatctggcacagatttcactctcaccatcaacagcctgcagcctgaagattttgcaacttattactgtctacaagattccaattacccgctcactttcggcggagggacacgactggagattaaaggtggcagcggacctaaatcttgtgacaaaactcacacatgcccaccgtgcccagcacctgaactcctggggggaccgtcagtcttcctcttccccccaaaacccaaggacaccctcatgatctcccggacccctgaggtcacatgcgtggtggtggacgtgagccacgaagaccctgaggtcaagttcaactggtacgtggacggcgtggaggtgcataatgccaagacaaagccgcgggaggagcagtacaacagcacgtaccgtgtggtcagcgtcctcaccgtcctgcaccaggactggctgaatggcaaggagtacaagtgcaaggtctccaacaaagccctcccagcccccatcgagaaaaccatctccaaagccaaagggcagccccgagaaccacaggtgtacaccctgcccccatcccgggatgagctgaccaagaaccaggtcagcctgacgtgcctggtcaaaggcttctatcccagcgacatcgccgtggagtgggagagcaatgggcagccggagaacaactacaagaccacgcctcccgtgctggactccgacggctccttcttcctctacagcaagctcaccgtggacaagagcagatggcagcaggggaacgtcttctcatgctccgtgatgcatgaggctctgcacaaccactacacgcagaagagcctctccctgtctccgggtaaatagtag

SEQ ID NO: 18 - protein, 112 aa, Homo sapiens
ALDTNYCFSSTEKNCCVRQLYIDFRKDLGWKWIHEPKGYHANFCLGPCPYIWSLDTQYSKVLALYNQHNPGASAAPCCVPQALEPLPIVYYVGRKPKVEQLSNMIVRSCKCS

SEQ ID NO: 19 - protein, 5 aa, Homo sapiens
GSSGG

SEQ ID NO: 20 - protein, 4 aa, Homo sapiens
GGSG

SEQ ID NO: 21 - protein, 5 aa, Homo sapiens
CPPCP

SEQ ID NO: 22 - protein, 5 aa, Homo sapiens
SYGMH

SEQ ID NO: 23 - protein, 17 aa, Homo sapiens
VISYDGSIKYYADSVKG

SEQ ID NO: 24 - protein, 14 aa, Homo sapiens
TGEYSGYDTSGVEL

SEQ ID NO: 25 - protein, 14 aa, Homo sapiens
TGEYSGYDTDPQYS

SEQ ID NO: 26 - protein, 14 aa, Homo sapiens
TGFYSGYDTPASPD

SEQ ID NO: 27 - protein, 11 aa, Homo sapiens
RASQGIGDDLG

SEQ ID NO: 28 - protein, 7 aa, Homo sapiens
GTSTLQS

SEQ ID NO: 29 - protein, 9 aa, Homo sapiens
LQDSNYPLT

SEQ ID NO: 30 - protein, 14 aa, Homo sapiens
  misc_feature (3)..(3): Xaa can be any naturally occurring amino acid
  misc_feature (10)..(14): Xaa can be any naturally occurring amino acid
TGXYSGYDTXXXXX